European Patent Application EP 4 537 821 A1, published April 16, 2025. Title: SRE-PTPRZ1抑制剂在制备治疗鳞状细胞癌的药物中的用途. Applicant: 四川大学华西医院. The sequence listing filed with the application follows.

SEQUENCE LISTING (4 sequences)

SEQ ID NO: 1 - DNA, 25 bp, synthetic construct
  source 1..25: mol_type = other DNA
cagccagtaaaaatgacttcagagc

SEQ ID NO: 2 - DNA, 19 bp, synthetic construct
  source 1..19: mol_type = other DNA
agagctgcagcaagactcg

SEQ ID NO: 3 - DNA, 21 bp, synthetic construct
  source 1..21: mol_type = other DNA
tgcgaatcctaaagcgtttcc

SEQ ID NO: 4 - DNA, 20 bp, synthetic construct
  source 1..20: mol_type = other DNA
tccattagcccaatccaggc